European Patent Application EP 4 596 565 A2, published August 6, 2025. Title: RNA-GUIDED TRANSCRIPTIONAL REGULATION. Applicant: President and Fellows of Harvard College. Application EP 22189419.9, filed August 9, 2022. The sequence listing filed with the application follows.

SEQUENCE LISTING (184 sequences)

SEQ ID NO: 1 - protein, 1368 aa, Streptococcus pyogenes [sequence omitted]

SEQ ID NO: 2 - DNA, 4332 bp, synthetic construct
  misc_feature 1..4332: note = VP64-activator construct
  source 1..4332: mol_type = other DNA
gccaccatggacaagaagtactccattgggctcgctatcggcacaaacagcgtcggctgggccgtcattacggacgagtacaaggtgccgagcaaaaaattcaaagttctgggcaataccgatcgccacagcataaagaagaacctcattggcgccctcctgttcgactccggggagacggccgaagccacgcggctcaaaagaacagcacggcgcagatatacccgcagaaagaatcggatctgctacctgcaggagatctttagtaatgagatggctaaggtggatgactctttcttccataggctggaggagtcctttttggtggaggaggataaaaagcacgagcgccacccaatctttggcaatatcgtggacgaggtggcgtaccatgaaaagtacccaaccatatatcatctgaggaagaagcttgtagacagtactgataaggctgacttgcggttgatctatctcgcgctggcgcatatgatcaaatttcggggacacttcctcatcgagggggacctgaacccagacaacagcgatgtcgacaaactctttatccaactggttcagacttacaatcagcttttcgaagagaacccgatcaacgcatccggagttgacgccaaagcaatcctgagcgctaggctgtccaaatcccggcggctcgaaaacctcatcgcacagctccctggggagaagaagaacggcctgtttggtaatcttatcgccctgtcactcgggctgacccccaactttaaatctaacttcgacctggccgaagatgccaagcttcaactgagcaaagacacctacgatgatgatctcgacaatctgctggcccagatcggcgaccagtacgcagacctttttttggcggcaaagaacctgtcagacgccattctgctgagtgatattctgcgagtgaacacggagatcaccaaagctccgctgagcgctagtatgatcaagcgctatgatgagcaccaccaagacttgactttgctgaaggcccttgtcagacagcaactgcctgagaagtacaaggaaattttcttcgatcagtctaaaaatggctacgccggatacattgacggcggagcaagccaggaggaattttacaaatttattaagcccatcttggaaaaaatggacggcaccgaggagctgctggtaaagcttaacagagaagatctgttgcgcaaacagcgcactttcgacaatggaagcatcccccaccagattcacctgggcgaactgcacgctatcctcaggcggcaagaggatttctacccctttttgaaagataacagggaaaagattgagaaaatcctcacatttcggataccctactatgtaggccccctcgcccggggaaattccagattcgcgtggatgactcgcaaatcagaagagaccatcactccctggaacttcgaggaagtcgtggataagggggcctctgcccagtccttcatcgaaaggatgactaactttgataaaaatctgcctaacgaaaaggtgcttcctaaacactctctgctgtacgagtacttcacagtttataacgagctcaccaaggtcaaatacgtcacagaagggatgagaaagccagcattcctgtctggagagcagaagaaagctatcgtggacctcctcttcaagacgaaccggaaagttaccgtgaaacagctcaaagaagactatttcaaaaagattgaatgtttcgactctgttgaaatcagcggagtggaggatcgcttcaacgcatccctgggaacgtatcacgatctcctgaaaatcattaaagacaaggacttcctggacaatgaggagaacgaggacattcttgaggacattgtcctcacccttacgttgtttgaagatagggagatgattgaagaacgcttgaaaacttacgctcatctcttcgacgacaaagtcatgaaacagctcaagaggcgccgatatacaggatgggggcggctgtcaagaaaactgatcaatgggatccgagacaagcagagtggaaagacaatcctggattttcttaagtccgatggatttgccaaccggaacttcatgcagttgatccatgatgactctctcacctttaaggaggacatccagaaagcacaagtttctggccagggggacagtcttcacgagcacatcgctaatcttgcaggtagcccagctatcaaaaagggaatactgcagaccgttaaggtcgtggatgaactcgtcaaagtaatgggaaggcataagcccgagaatatcgttatcgagatggcccgagagaaccaaactacccagaagggacagaagaacagtagggaaaggatgaagaggattgaagagggtataaaagaactggggtcccaaatccttaaggaacacccagttgaaaacacccagcttcagaatgagaagctctacctgtactacctgcagaacggcagggacatgtacgtggatcaggaactggacatcaatcggctctccgactacgacgtggctgctatcgtgccccagtcttttctcaaagatgattctattgataataaagtgttgacaagatccgataaagctagagggaagagtgataacgtcccctcagaagaagttgtcaagaaaatgaaaaattattggcggcagctgctgaacgccaaactgatcacacaacggaagttcgataatctgactaaggctgaacgaggtggcctgtctgagttggataaagccggcttcatcaaaaggcagcttgttgagacacgccagatcaccaagcacgtggcccaaattctcgattcacgcatgaacaccaagtacgatgaaaatgacaaactgattcgagaggtgaaagttattactctgaagtctaagctggtctcagatttcagaaaggactttcagttttataaggtgagagagatcaacaattaccaccatgcgcatgatgcctacctgaatgcagtggtaggcactgcacttatcaaaaaatatcccaagcttgaatctgaatttgtttacggagactataaagtgtacgatgttaggaaaatgatcgcaaagtctgagcaggaaataggcaaggccaccgctaagtacttcttttacagcaatattatgaattttttcaagaccgagattacactggccaatggagagattcggaagcgaccacttatcgaaacaaacggagaaacaggagaaatcgtgtgggacaagggtagggatttcgcgacagtccggaaggtcctgtccatgccgcaggtgaacatcgttaaaaagaccgaagtacagaccggaggcttctccaaggaaagtatcctcccgaaaaggaacagcgacaagctgatcgcacgcaaaaaagattgggaccccaagaaatacggcggattcgattctcctacagtcgcttacagtgtactggttgtggccaaagtggagaaagggaagtctaaaaaactcaaaagcgtcaaggaactgctgggcatcacaatcatggagcgatcaagcttcgaaaaaaaccccatcgactttctcgaggcgaaaggatataaagaggtcaaaaaagacctcatcattaagcttcccaagtactctctctttgagcttgaaaacggccggaaacgaatgctcgctagtgcgggcgagctgcagaaaggtaacgagctggcactgccctctaaatacgttaatttcttgtatctggccagccactatgaaaagctcaaagggtctcccgaagataatgagcagaagcagctgttcgtggaacaacacaaacactaccttgatgagatcatcgagcaaataagcgaattctccaaaagagtgatcctcgccgacgctaacctcgataaggtgctttctgcttacaataagcacagggataagcccatcagggagcaggcagaaaacattatccacttgtttactctgaccaacttgggcgcgcctgcagccttcaagtacttcgacaccaccatagacagaaagcggtacacctctacaaaggaggtcctggacgccacactgattcatcagtcaattacggggctctatgaaacaagaatcgacctctctcagctcggtggagacagcagggctgaccccaagaagaagaggaaggtggaggccagcggttccggacgggctgacgcattggacgattttgatctggatatgctgggaagtgacgccctcgatgattttgaccttgacatgcttggttcggatgcccttgatgactttgacctcgacatgctcggcagtgacgcccttgatgatttcgacctggacatgctgattaactctagatga

SEQ ID NO: 3 - DNA, 4365 bp, synthetic construct
  misc_feature 1..4365: note = VP64-activator construct
  source 1..4365: mol_type = other DNA
gccaccatgcccaagaagaagaggaaggtgggaagggggatggacaagaagtactccattgggctcgctatcggcacaaacagcgtcggctgggccgtcattacggacgagtacaaggtgccgagcaaaaaattcaaagttctgggcaataccgatcgccacagcataaagaagaacctcattggcgccctcctgttcgactccggggagacggccgaagccacgcggctcaaaagaacagcacggcgcagatatacccgcagaaagaatcggatctgctacctgcaggagatctttagtaatgagatggctaaggtggatgactctttcttccataggctggaggagtcctttttggtggaggaggataaaaagcacgagcgccacccaatctttggcaatatcgtggacgaggtggcgtaccatgaaaagtacccaaccatatatcatctgaggaagaagcttgtagacagtactgataaggctgacttgcggttgatctatctcgcgctggcgcatatgatcaaatttcggggacacttcctcatcgagggggacctgaacccagacaacagcgatgtcgacaaactctttatccaactggttcagacttacaatcagcttttcgaagagaacccgatcaacgcatccggagttgacgccaaagcaatcctgagcgctaggctgtccaaatcccggcggctcgaaaacctcatcgcacagctccctggggagaagaagaacggcctgtttggtaatcttatcgccctgtcactcgggctgacccccaactttaaatctaacttcgacctggccgaagatgccaagcttcaactgagcaaagacacctacgatgatgatctcgacaatctgctggcccagatcggcgaccagtacgcagacctttttttggcggcaaagaacctgtcagacgccattctgctgagtgatattctgcgagtgaacacggagatcaccaaagctccgctgagcgctagtatgatcaagcgctatgatgagcaccaccaagacttgactttgctgaaggcccttgtcagacagcaactgcctgagaagtacaaggaaattttcttcgatcagtctaaaaatggctacgccggatacattgacggcggagcaagccaggaggaattttacaaatttattaagcccatcttggaaaaaatggacggcaccgaggagctgctggtaaagcttaacagagaagatctgttgcgcaaacagcgcactttcgacaatggaagcatcccccaccagattcacctgggcgaactgcacgctatcctcaggcggcaagaggatttctacccctttttgaaagataacagggaaaagattgagaaaatcctcacatttcggataccctactatgtaggccccctcgcccggggaaattccagattcgcgtggatgactcgcaaatcagaagagaccatcactccctggaacttcgaggaagtcgtggataagggggcctctgcccagtccttcatcgaaaggatgactaactttgataaaaatctgcctaacgaaaaggtgcttcctaaacactctctgctgtacgagtacttcacagtttataacgagctcaccaaggtcaaatacgtcacagaagggatgagaaagccagcattcctgtctggagagcagaagaaagctatcgtggacctcctcttcaagacgaaccggaaagttaccgtgaaacagctcaaagaagactatttcaaaaagattgaatgtttcgactctgttgaaatcagcggagtggaggatcgcttcaacgcatccctgggaacgtatcacgatctcctgaaaatcattaaagacaaggacttcctggacaatgaggagaacgaggacattcttgaggacattgtcctcacccttacgttgtttgaagatagggagatgattgaagaacgcttgaaaacttacgctcatctcttcgacgacaaagtcatgaaacagctcaagaggcgccgatatacaggatgggggcggctgtcaagaaaactgatcaatgggatccgagacaagcagagtggaaagacaatcctggattttcttaagtccgatggatttgccaaccggaacttcatgcagttgatccatgatgactctctcacctttaaggaggacatccagaaagcacaagtttctggccagggggacagtcttcacgagcacatcgctaatcttgcaggtagcccagctatcaaaaagggaatactgcagaccgttaaggtcgtggatgaactcgtcaaagtaatgggaaggcataagcccgagaatatcgttatcgagatggcccgagagaaccaaactacccagaagggacagaagaacagtagggaaaggatgaagaggattgaagagggtataaaagaactggggtcccaaatccttaaggaacacccagttgaaaacacccagcttcagaatgagaagctctacctgtactacctgcagaacggcagggacatgtacgtggatcaggaactggacatcaatcggctctccgactacgacgtggctgctatcgtgccccagtcttttctcaaagatgattctattgataataaagtgttgacaagatccgataaagctagagggaagagtgataacgtcccctcagaagaagttgtcaagaaaatgaaaaattattggcggcagctgctgaacgccaaactgatcacacaacggaagttcgataatctgactaaggctgaacgaggtggcctgtctgagttggataaagccggcttcatcaaaaggcagcttgttgagacacgccagatcaccaagcacgtggcccaaattctcgattcacgcatgaacaccaagtacgatgaaaatgacaaactgattcgagaggtgaaagttattactctgaagtctaagctggtctcagatttcagaaaggactttcagttttataaggtgagagagatcaacaattaccaccatgcgcatgatgcctacctgaatgcagtggtaggcactgcacttatcaaaaaatatcccaagcttgaatctgaatttgtttacggagactataaagtgtacgatgttaggaaaatgatcgcaaagtctgagcaggaaataggcaaggccaccgctaagtacttcttttacagcaatattatgaattttttcaagaccgagattacactggccaatggagagattcggaagcgaccacttatcgaaacaaacggagaaacaggagaaatcgtgtgggacaagggtagggatttcgcgacagtccggaaggtcctgtccatgccgcaggtgaacatcgttaaaaagaccgaagtacagaccggaggcttctccaaggaaagtatcctcccgaaaaggaacagcgacaagctgatcgcacgcaaaaaagattgggaccccaagaaatacggcggattcgattctcctacagtcgcttacagtgtactggttgtggccaaagtggagaaagggaagtctaaaaaactcaaaagcgtcaaggaactgctgggcatcacaatcatggagcgatcaagcttcgaaaaaaaccccatcgactttctcgaggcgaaaggatataaagaggtcaaaaaagacctcatcattaagcttcccaagtactctctctttgagcttgaaaacggccggaaacgaatgctcgctagtgcgggcgagctgcagaaaggtaacgagctggcactgccctctaaatacgttaatttcttgtatctggccagccactatgaaaagctcaaagggtctcccgaagataatgagcagaagcagctgttcgtggaacaacacaaacactaccttgatgagatcatcgagcaaataagcgaattctccaaaagagtgatcctcgccgacgctaacctcgataaggtgctttctgcttacaataagcacagggataagcccatcagggagcaggcagaaaacattatccacttgtttactctgaccaacttgggcgcgcctgcagccttcaagtacttcgacaccaccatagacagaaagcggtacacctctacaaaggaggtcctggacgccacactgattcatcagtcaattacggggctctatgaaacaagaatcgacctctctcagctcggtggagacagcagggctgaccccaagaagaagaggaaggtggaggccagcggttccggacgggctgacgcattggacgattttgatctggatatgctgggaagtgacgccctcgatgattttgaccttgacatgcttggttcggatgcccttgatgactttgacctcgacatgctcggcagtgacgcccttgatgatttcgacctggacatgctgattaactctagatga

SEQ ID NO: 4 - DNA, 4425 bp, synthetic construct
  misc_feature 1..4425: note = VP64-activator construct
  source 1..4425: mol_type = other DNA
gccaccatggacaagaagtactccattgggctcgctatcggcacaaacagcgtcggctgggccgtcattacggacgagtacaaggtgccgagcaaaaaattcaaagttctgggcaataccgatcgccacagcataaagaagaacctcattggcgccctcctgttcgactccggggagacggccgaagccacgcggctcaaaagaacagcacggcgcagatatacccgcagaaagaatcggatctgctacctgcaggagatctttagtaatgagatggctaaggtggatgactctttcttccataggctggaggagtcctttttggtggaggaggataaaaagcacgagcgccacccaatctttggcaatatcgtggacgaggtggcgtaccatgaaaagtacccaaccatatatcatctgaggaagaagcttgtagacagtactgataaggctgacttgcggttgatctatctcgcgctggcgcatatgatcaaatttcggggacacttcctcatcgagggggacctgaacccagacaacagcgatgtcgacaaactctttatccaactggttcagacttacaatcagcttttcgaagagaacccgatcaacgcatccggagttgacgccaaagcaatcctgagcgctaggctgtccaaatcccggcggctcgaaaacctcatcgcacagctccctggggagaagaagaacggcctgtttggtaatcttatcgccctgtcactcgggctgacccccaactttaaatctaacttcgacctggccgaagatgccaagcttcaactgagcaaagacacctacgatgatgatctcgacaatctgctggcccagatcggcgaccagtacgcagacctttttttggcggcaaagaacctgtcagacgccattctgctgagtgatattctgcgagtgaacacggagatcaccaaagctccgctgagcgctagtatgatcaagcgctatgatgagcaccaccaagacttgactttgctgaaggcccttgtcagacagcaactgcctgagaagtacaaggaaattttcttcgatcagtctaaaaatggctacgccggatacattgacggcggagcaagccaggaggaattttacaaatttattaagcccatcttggaaaaaatggacggcaccgaggagctgctggtaaagcttaacagagaagatctgttgcgcaaacagcgcactttcgacaatggaagcatcccccaccagattcacctgggcgaactgcacgctatcctcaggcggcaagaggatttctacccctttttgaaagataacagggaaaagattgagaaaatcctcacatttcggataccctactatgtaggccccctcgcccggggaaattccagattcgcgtggatgactcgcaaatcagaagagaccatcactccctggaacttcgaggaagtcgtggataagggggcctctgcccagtccttcatcgaaaggatgactaactttgataaaaatctgcctaacgaaaaggtgcttcctaaacactctctgctgtacgagtacttcacagtttataacgagctcaccaaggtcaaatacgtcacagaagggatgagaaagccagcattcctgtctggagagcagaagaaagctatcgtggacctcctcttcaagacgaaccggaaagttaccgtgaaacagctcaaagaagactatttcaaaaagattgaatgtttcgactctgttgaaatcagcggagtggaggatcgcttcaacgcatccctgggaacgtatcacgatctcctgaaaatcattaaagacaaggacttcctggacaatgaggagaacgaggacattcttgaggacattgtcctcacccttacgttgtttgaagatagggagatgattgaagaacgcttgaaaacttacgctcatctcttcgacgacaaagtcatgaaacagctcaagaggcgccgatatacaggatgggggcggctgtcaagaaaactgatcaatgggatccgagacaagcagagtggaaagacaatcctggattttcttaagtccgatggatttgccaaccggaacttcatgcagttgatccatgatgactctctcacctttaaggaggacatccagaaagcacaagtttctggccagggggacagtcttcacgagcacatcgctaatcttgcaggtagcccagctatcaaaaagggaatactgcagaccgttaaggtcgtggatgaactcgtcaaagtaatgggaaggcataagcccgagaatatcgttatcgagatggcccgagagaaccaaactacccagaagggacagaagaacagtagggaaaggatgaagaggattgaagagggtataaaagaactggggtcccaaatccttaaggaacacccagttgaaaacacccagcttcagaatgagaagctctacctgtactacctgcagaacggcagggacatgtacgtggatcaggaactggacatcaatcggctctccgactacgacgtggctgctatcgtgccccagtcttttctcaaagatgattctattgataataaagtgttgacaagatccgataaagctagagggaagagtgataacgtcccctcagaagaagttgtcaagaaaatgaaaaattattggcggcagctgctgaacgccaaactgatcacacaacggaagttcgataatctgactaaggctgaacgaggtggcctgtctgagttggataaagccggcttcatcaaaaggcagcttgttgagacacgccagatcaccaagcacgtggcccaaattctcgattcacgcatgaacaccaagtacgatgaaaatgacaaactgattcgagaggtgaaagttattactctgaagtctaagctggtctcagatttcagaaaggactttcagttttataaggtgagagagatcaacaattaccaccatgcgcatgatgcctacctgaatgcagtggtaggcactgcacttatcaaaaaatatcccaagcttgaatctgaatttgtttacggagactataaagtgtacgatgttaggaaaatgatcgcaaagtctgagcaggaaataggcaaggccaccgctaagtacttcttttacagcaatattatgaattttttcaagaccgagattacactggccaatggagagattcggaagcgaccacttatcgaaacaaacggagaaacaggagaaatcgtgtgggacaagggtagggatttcgcgacagtccggaaggtcctgtccatgccgcaggtgaacatcgttaaaaagaccgaagtacagaccggaggcttctccaaggaaagtatcctcccgaaaaggaacagcgacaagctgatcgcacgcaaaaaagattgggaccccaagaaatacggcggattcgattctcctacagtcgcttacagtgtactggttgtggccaaagtggagaaagggaagtctaaaaaactcaaaagcgtcaaggaactgctgggcatcacaatcatggagcgatcaagcttcgaaaaaaaccccatcgactttctcgaggcgaaaggatataaagaggtcaaaaaagacctcatcattaagcttcccaagtactctctctttgagcttgaaaacggccggaaacgaatgctcgctagtgcgggcgagctgcagaaaggtaacgagctggcactgccctctaaatacgttaatttcttgtatctggccagccactatgaaaagctcaaagggtctcccgaagataatgagcagaagcagctgttcgtggaacaacacaaacactaccttgatgagatcatcgagcaaataagcgaattctccaaaagagtgatcctcgccgacgctaacctcgataaggtgctttctgcttacaataagcacagggataagcccatcagggagcaggcagaaaacattatccacttgtttactctgaccaacttgggcgcgcctgcagccttcaagtacttcgacaccaccatagacagaaagcggtacacctctacaaaggaggtcctggacgccacactgattcatcagtcaattacggggctctatgaaacaagaatcgacctctctcagctcggtggagacagcagggctgaccccaagaagaagaggaaggtggaggccagcggttccggacgggctgacgcattggacgattttgatctggatatgctgggaagtgacgccctcgatgattttgaccttgacatgcttggttcggatgcccttgatgactttgacctcgacatgctcggcagtgacgcccttgatgatttcgacctggacatgctgattaactctagagcggccgcagatccaaaaaagaagagaaaggtagatccaaaaaagaagagaaaggtagatccaaaaaagaagagaaaggtagatacggccgcatag

SEQ ID NO: 5 - DNA, 587 bp, synthetic construct
  misc_feature 1..587: note = MS2-activator construct
  source 1..587: mol_type = other DNA
ccaccatgggacctaagaaaaagaggaaggtggcggccgcttctagaatggcttctaactttactcagttcgttctcgtcgacaatggcggaactggcgacgtgactgtcgccccaagcaacttcgctaacgggatcgctgaatggatcagctctaactcgcgttcacaggcttacaaagtaacctgtagcgttcgtcagagctctgcgcagaatcgcaaatacaccatcaaagtcgaggtgcctaaaggcgcctggcgttcgtacttaaatatggaactaaccattccaattttcgccacgaattccgactgcgagcttattgttaaggcaatgcaaggtctcctaaaagatggaaacccgattccctcagcaatcgcagcaaactccggcatctacgaggccagcggttccggacgggctgacgcattggacgattttgatctggatatgctgggaagtgacgccctcgatgattttgaccttgacatgcttggttcggatgcccttgatgactttgacctcgacatgctcggcagtgacgcccttgatgatttcgacctggacatgctgattaactctagatga

SEQ ID NO: 6 - DNA, 681 bp, synthetic construct
  misc_feature 1..681: note = MS2-activator construct
  source 1..681: mol_type = other DNA
gccaccatgggacctaagaaaaagaggaaggtggcggccgcttctagaatggcttctaactttactcagttcgttctcgtcgacaatggcggaactggcgacgtgactgtcgccccaagcaacttcgctaacgggatcgctgaatggatcagctctaactcgcgttcacaggcttacaaagtaacctgtagcgttcgtcagagctctgcgcagaatcgcaaatacaccatcaaagtcgaggtgcctaaaggcgcctggcgttcgtacttaaatatggaactaaccattccaattttcgccacgaattccgactgcgagcttattgttaaggcaatgcaaggtctcctaaaagatggaaacccgattccctcagcaatcgcagcaaactccggcatctacgaggccagcggttccggacgggctgacgcattggacgattttgatctggatatgctgggaagtgacgccctcgatgattttgaccttgacatgcttggttcggatgcccttgatgactttgacctcgacatgctcggcagtgacgcccttgatgatttcgacctggacatgctgattaactctagagcggccgcagatccaaaaaagaagagaaaggtagatccaaaaaagaagagaaaggtagatccaaaaaagaagagaaaggtagatacggccgcatag

SEQ ID NO: 7 - DNA, 557 bp, synthetic construct
  misc_feature 1..557: note = MS2-activator construct
  misc_feature 320..339: note = wherein N is G, A, T or C
  source 1..557: mol_type = other DNA
tgtacaaaaaagcaggctttaaaggaaccaattcagtcgactggatccggtaccaaggtcgggcaggaagagggcctatttcccatgattccttcatatttgcatatacgatacaaggctgttagagagataattagaattaatttgactgtaaacacaaagatattagtacaaaatacgtgacgtagaaagtaataatttcttgggtagtttgcagttttaaaattatgttttaaaatggactatcatatgcttaccgtaacttgaaagtatttcgatttcttggctttatatatcttgtggaaaggacgaaacaccgnnnnnnnnnnnnnnnnnnnngttttagagctagaaatagcaagttaaaataaggctagtccgttatcaacttgaaaaagtggcaccgagtcggtgctctgcaggtcgactctagaaaacatgaggatcacccatgtctgcagtattcccgggttcattagatcctaaggtacctaattgcctagaaaacatgaggatcacccatgtctgcaggtcgactctagaaattttttctagac

SEQ ID NO: 8 - DNA, 882 bp, synthetic construct
  misc_feature 1..882: note = Activation reporter construct
  source 1..882: mol_type = other DNA
tagggataacagggtaatagtgtcccctccaccccacagtggggcgaggtaggcgtgtacggtgggaggcctatataagcagagctcgtttagtgaaccgtcagatcgcctggagaattcgccaccatggactacaaggatgacgacgataaaacttccggtggcggactgggttccaccgtgagcaagggcgaggaggtcatcaaagagttcatgcgcttcaaggtgcgcatggagggctccatgaacggccacgagttcgagatcgagggcgagggcgagggccgcccctacgagggcacccagaccgccaagctgaaggtgaccaagggcggccccctgcccttcgcctgggacatcctgtccccccagttcatgtacggctccaaggcgtacgtgaagcaccccgccgacatccccgattacaagaagctgtccttccccgagggcttcaagtgggagcgcgtgatgaacttcgaggacggcggtctggtgaccgtgacccaggactcctccctgcaggacggcacgctgatctacaaggtgaagatgcgcggcaccaacttcccccccgacggccccgtaatgcagaagaagaccatgggctgggaggcctccaccgagcgcctgtacccccgcgacggcgtgctgaagggcgagatccaccaggccctgaagctgaaggacggcggccactacctggtggagttcaagaccatctacatggccaagaagcccgtgcaactgcccggctactactacgtggacaccaagctggacatcacctcccacaacgaggactacaccatcgtggaacagtacgagcgctccgagggccgccaccacctgttcctgtacggcatggacgagctgtacaagtaa

SEQ ID NO: 9 - DNA, 882 bp, synthetic construct
  misc_feature 1..882: note = Activation reporter construct
  source 1..882: mol_type = other DNA
tagggataacagggtaatagtggggccactagggacaggattggcgaggtaggcgtgtacggtgggaggcctatataagcagagctcgtttagtgaaccgtcagatcgcctggagaattcgccaccatggactacaaggatgacgacgataaaacttccggtggcggactgggttccaccgtgagcaagggcgaggaggtcatcaaagagttcatgcgcttcaaggtgcgcatggagggctccatgaacggccacgagttcgagatcgagggcgagggcgagggccgcccctacgagggcacccagaccgccaagctgaaggtgaccaagggcggccccctgcccttcgcctgggacatcctgtccccccagttcatgtacggctccaaggcgtacgtgaagcaccccgccgacatccccgattacaagaagctgtccttccccgagggcttcaagtgggagcgcgtgatgaacttcgaggacggcggtctggtgaccgtgacccaggactcctccctgcaggacggcacgctgatctacaaggtgaagatgcgcggcaccaacttcccccccgacggccccgtaatgcagaagaagaccatgggctgggaggcctccaccgagcgcctgtacccccgcgacggcgtgctgaagggcgagatccaccaggccctgaagctgaaggacggcggccactacctggtggagttcaagaccatctacatggccaagaagcccgtgcaactgcccggctactactacgtggacaccaagctggacatcacctcccacaacgaggactacaccatcgtggaacagtacgagcgctccgagggccgccaccacctgttcctgtacggcatggacgagctgtacaagtaa

SEQ ID NO: 10 - DNA, 912 bp, synthetic construct
  misc_feature 1..912: note = Specificity reporter library
  misc_feature 22..44: note = wherein N is G, A, T or C
  misc_feature 154..177: note = wherein N is G, A, T or C
  source 1..912: mol_type = other DNA
tagggataacagggtaatagtnnnnnnnnnnnnnnnnnnnnnnncgaggtaggcgtgtacggtgggaggcctatataagcagagctcgtttagtgaaccgtcagatcgcctggagaattcgccaccatggactacaaggatgacgacgataaannnnnnnnnnnnnnnnnnnnnnnnacttccggtggcggactgggttccaccgtgagcaagggcgaggaggtcatcaaagagttcatgcgcttcaaggtgcgcatggagggctccatgaacggccacgagttcgagatcgagggcgagggcgagggccgcccctacgagggcacccagaccgccaagctgaaggtgaccaagggcggccccctgcccttcgcctgggacatcctgtccccccagttcatgtacggctccaaggcgtacgtgaagcaccccgccgacatccccgattacaagaagctgtccttccccgagggcttcaagtgggagcgcgtgatgaacttcgaggacggcggtctggtgaccgtgacccaggactcctccctgcaggacggcacgctgatctacaaggtgaagatgcgcggcaccaacttcccccccgacggccccgtaatgcagaagaagaccatgggctgggaggcctccaccgagcgcctgtacccccgcgacggcgtgctgaagggcgagatccaccaggccctgaagctgaaggacggcggccactacctggtggagttcaagaccatctacatggccaagaagcccgtgcaactgcccggctactactacgtggacaccaagctggacatcacctcccacaacgaggactacaccatcgtggaacagtacgagcgctccgagggccgccaccacctgttcctgtacggcatggacgagctgtacaagtaagaattc

SEQ ID NO: 11 - DNA, 23 bp, synthetic construct
  misc_feature 1..23: note = Target probe
  source 1..23: mol_type = other DNA
ctggcggatcactcgcggttagg

SEQ ID NO: 12 - DNA, 23 bp, synthetic construct
  misc_feature 1..23: note = Target probe
  source 1..23: mol_type = other DNA
cctcggcctccaaaagtgctagg

SEQ ID NO: 13 - DNA, 23 bp, synthetic construct
  misc_feature 1..23: note = Target probe
  source 1..23: mol_type = other DNA
acgctgattcctgcagatcaggg

SEQ ID NO: 14 - DNA, 23 bp, synthetic construct
  misc_feature 1..23: note = Target probe
  source 1..23: mol_type = other DNA
ccaggaatacgtatccaccaggg

SEQ ID NO: 15 - DNA, 23 bp, synthetic construct
  misc_feature 1..23: note = Target probe
  source 1..23: mol_type = other DNA
gccacacccaagcgatcaaatgg

SEQ ID NO: 16 - DNA, 23 bp, synthetic construct
  misc_feature 1..23: note = Target probe
  source 1..23: mol_type = other DNA
aaataatacattctaaggtaagg

SEQ ID NO: 17 - DNA, 23 bp, synthetic construct
  misc_feature 1..23: note = Target probe
  source 1..23: mol_type = other DNA
gctactggggaggctgaggcagg

SEQ ID NO: 18 - DNA, 23 bp, synthetic construct
  misc_feature 1..23: note = Target probe
  source 1..23: mol_type = other DNA
tagcaatacagtcacattaatgg

SEQ ID NO: 19 - DNA, 23 bp, synthetic construct
  misc_feature 1..23: note = Target probe
  source 1..23: mol_type = other DNA
ctcatgtgatccccccgtctcgg

SEQ ID NO: 20 - DNA, 23 bp, synthetic construct
  misc_feature 1..23: note = Target probe
  source 1..23: mol_type = other DNA
ccgggcagagagtgaacgcgcgg

SEQ ID NO: 21 - DNA, 23 bp, synthetic construct
  misc_feature 1..23: note = Target probe
  source 1..23: mol_type = other DNA
ttccttccctctcccgtgcttgg

SEQ ID NO: 22 - DNA, 23 bp, synthetic construct
  misc_feature 1..23: note = Target probe
  source 1..23: mol_type = other DNA
tctctgcaaagcccctggagagg

SEQ ID NO: 23 - DNA, 23 bp, synthetic construct
  misc_feature 1..23: note = Target probe
  source 1..23: mol_type = other DNA
aatgcagttgccgagtgcagtgg

SEQ ID NO: 24 - DNA, 23 bp, synthetic construct
  misc_feature 1..23: note = Target probe
  source 1..23: mol_type = other DNA
cctcagcctcctaaagtgctggg

SEQ ID NO: 25 - DNA, 23 bp, synthetic construct
  misc_feature 1..23: note = Target probe
  source 1..23: mol_type = other DNA
gagtccaaatcctctttactagg

SEQ ID NO: 26 - DNA, 23 bp, synthetic construct
  misc_feature 1..23: note = Target probe
  source 1..23: mol_type = other DNA
gagtgtctggatttgggataagg

SEQ ID NO: 27 - DNA, 23 bp, synthetic construct
  misc_feature 1..23: note = Target probe
  source 1..23: mol_type = other DNA
cagcacctcatctcccagtgagg

SEQ ID NO: 28 - DNA, 23 bp, synthetic construct
  misc_feature 1..23: note = Target probe
  source 1..23: mol_type = other DNA
tctaaaacccagggaatcatggg

SEQ ID NO: 29 - DNA, 23 bp, synthetic construct
  misc_feature 1..23: note = Target probe
  source 1..23: mol_type = other DNA
cacaaggcagccagggatccagg

SEQ ID NO: 30 - DNA, 23 bp, synthetic construct
  misc_feature 1..23: note = Target probe
  source 1..23: mol_type = other DNA
gatggcaagctgagaaacactgg

SEQ ID NO: 31 - DNA, 23 bp, synthetic construct
  misc_feature 1..23: note = Target probe
  source 1..23: mol_type = other DNA
tgaaatgcacgcatacaattagg

SEQ ID NO: 32 - DNA, 23 bp, synthetic construct
  misc_feature 1..23: note = Target probe
  source 1..23: mol_type = other DNA
ccagtccagacctggccttctgg

SEQ ID NO: 33 - DNA, 23 bp, synthetic construct
  misc_feature 1..23: note = Target probe
  source 1..23: mol_type = other DNA
cccagaaaaacagaccctgaagg

SEQ ID NO: 34 - DNA, 23 bp, synthetic construct
  misc_feature 1..23: note = Target probe
  source 1..23: mol_type = other DNA
aagggttgagcacttgtttaggg

SEQ ID NO: 35 - DNA, 23 bp, synthetic construct
  misc_feature 1..23: note = Target probe
  source 1..23: mol_type = other DNA
atgtctgagttttggttgagagg

SEQ ID NO: 36 - DNA, 23 bp, synthetic construct
  misc_feature 1..23: note = Target probe
  source 1..23: mol_type = other DNA
ggtcccttgaaggggaagtaggg

SEQ ID NO: 37 - DNA, 23 bp, synthetic construct
  misc_feature 1..23: note = Target probe
  source 1..23: mol_type = other DNA
tggcagtctactcttgaagatgg

SEQ ID NO: 38 - DNA, 23 bp, synthetic construct
  misc_feature 1..23: note = Target probe
  source 1..23: mol_type = other DNA
ggcacagtgccagaggtctgtgg

SEQ ID NO: 39 - DNA, 23 bp, synthetic construct
  misc_feature 1..23: note = Target probe
  source 1..23: mol_type = other DNA
taaaaataaaaaaactaacaggg

SEQ ID NO: 40 - DNA, 23 bp, synthetic construct
  misc_feature 1..23: note = Target probe
  source 1..23: mol_type = other DNA
tctgtgggggacctgcactgagg

SEQ ID NO: 41 - DNA, 23 bp, synthetic construct
  misc_feature 1..23: note = Target probe
  source 1..23: mol_type = other DNA
ggccagaggtcaaggctagtggg

SEQ ID NO: 42 - DNA, 23 bp, synthetic construct
  misc_feature 1..23: note = Target probe
  source 1..23: mol_type = other DNA
cacgaccgaaacccttcttacgg

SEQ ID NO: 43 - DNA, 23 bp, synthetic construct
  misc_feature 1..23: note = Target probe
  source 1..23: mol_type = other DNA
gttgaatgaagacagtctagtgg

SEQ ID NO: 44 - DNA, 23 bp, synthetic construct
  misc_feature 1..23: note = Target probe
  source 1..23: mol_type = other DNA
taagaacagagcaagttacgtgg

SEQ ID NO: 45 - DNA, 23 bp, synthetic construct
  misc_feature 1..23: note = Target probe
  source 1..23: mol_type = other DNA
tgtaaggtaagagaggagagcgg

SEQ ID NO: 46 - DNA, 23 bp, synthetic construct
  misc_feature 1..23: note = Target probe
  source 1..23: mol_type = other DNA
tgacacaccaactcctgcactgg

SEQ ID NO: 47 - DNA, 23 bp, synthetic construct
  misc_feature 1..23: note = Target probe
  source 1..23: mol_type = other DNA
tttacccacttccttcgaaaagg

SEQ ID NO: 48 - DNA, 23 bp, synthetic construct
  misc_feature 1..23: note = Target probe
  source 1..23: mol_type = other DNA
gtggctggcaggctggctctggg

SEQ ID NO: 49 - DNA, 23 bp, synthetic construct
  misc_feature 1..23: note = Target probe
  source 1..23: mol_type = other DNA
ctcccccggcctcccccgcgcgg

SEQ ID NO: 50 - DNA, 23 bp, synthetic construct
  misc_feature 1..23: note = Target probe
  source 1..23: mol_type = other DNA
caaaacccggcagcgaggctggg

SEQ ID NO: 51 - DNA, 23 bp, synthetic construct
  misc_feature 1..23: note = Target probe
  source 1..23: mol_type = other DNA
aggagccgccgcgcgctgattgg

SEQ ID NO: 52 - DNA, 23 bp, synthetic construct
  misc_feature 1..23: note = Target probe
  source 1..23: mol_type = other DNA
cacacacacccacacgagatggg

SEQ ID NO: 53 - DNA, 23 bp, synthetic construct
  misc_feature 1..23: note = Target probe
  source 1..23: mol_type = other DNA
gaagaagctaaagagccagaggg

SEQ ID NO: 54 - DNA, 23 bp, synthetic construct
  misc_feature 1..23: note = Target probe
  source 1..23: mol_type = other DNA
atgagaatttcaataacctcagg

SEQ ID NO: 55 - DNA, 23 bp, synthetic construct
  misc_feature 1..23: note = Target probe
  source 1..23: mol_type = other DNA
tcccgctctgttgcccaggctgg

SEQ ID NO: 56 - DNA, 23 bp, synthetic construct
  misc_feature 1..23: note = Target probe
  source 1..23: mol_type = other DNA
cagacacccaccaccatgcgtgg

SEQ ID NO: 57 - DNA, 23 bp, synthetic construct
  misc_feature 1..23: note = Target probe
  source 1..23: mol_type = other DNA
tcccaatttactgggattacagg

SEQ ID NO: 58 - DNA, 23 bp, synthetic construct
  misc_feature 1..23: note = Target probe
  source 1..23: mol_type = other DNA
tgatttaaaagttggaaacgtgg

SEQ ID NO: 59 - DNA, 23 bp, synthetic construct
  misc_feature 1..23: note = Target probe
  source 1..23: mol_type = other DNA
tctagttccccacctagtctggg

SEQ ID NO: 60 - DNA, 23 bp, synthetic construct
  misc_feature 1..23: note = Target probe
  source 1..23: mol_type = other DNA
gattaactgagaattcacaaggg

SEQ ID NO: 61 - DNA, 23 bp, synthetic construct
  misc_feature 1..23: note = Target probe
  source 1..23: mol_type = other DNA
cgccaggaggggtgggtctaagg

SEQ ID NO: 62 - DNA, 23 bp, synthetic construct
  misc_feature 1..23: note = Reporter construct
  source 1..23: mol_type = other DNA
gtcccctccaccccacagtgggg

SEQ ID NO: 63 - DNA, 23 bp, synthetic construct
  misc_feature 1..23: note = Reporter construct
  source 1..23: mol_type = other DNA
ggggccactagggacaggattgg

SEQ ID NO: 64 - DNA, 71 bp, synthetic construct
  misc_feature 1..71: note = Target oligonucleotide sequence
  source 1..71: mol_type = other DNA
taatacttttatctgtcccctccaccccacagtggggccactagggacaggattggtgacagaaaagcccc

SEQ ID NO: 65 - DNA, 20 bp, synthetic construct
  misc_feature 1..20: note = Target oligonucleotide sequence
  source 1..20: mol_type = other DNA
ggggccactagggacaggat

SEQ ID NO: 66 - RNA, 80 nt, synthetic construct
  misc_feature 1..80: note = Guide RNA
  source 1..80: mol_type = other RNA
gttttagagctagaaatagcaagttaaaataaggctagcttgttatcaacttgaaaaagtggcaccgagtcggtgctttt

SEQ ID NO: 67 - DNA, 23 bp, synthetic construct
  misc_feature 1..23: note = Target oligonucleotide sequence
  source 1..23: mol_type = other DNA
gtcccctccaccccacagtgcag

SEQ ID NO: 68 - DNA, 23 bp, synthetic construct
  misc_feature 1..23: note = Target oligonucleotide sequence
  source 1..23: mol_type = other DNA
gtcccctccaccccacagtgcaa

SEQ ID NO: 69 - DNA, 23 bp, synthetic construct
  misc_feature 1..23: note = Target oligonucleotide sequence
  source 1..23: mol_type = other DNA
gtcccctccaccccacagtgcgg

SEQ ID NO: 70 - DNA, 52 bp, synthetic construct
  misc_feature 1..52: note = Target oligonucleotide sequence
  source 1..52: mol_type = other DNA
tgtcccctccaccccacagtggggccactagggacaggattggtgacagaaa

SEQ ID NO: 71 - DNA, 52 bp, synthetic construct
  misc_feature 1..52: note = Target oligonucleotide sequence
  source 1..52: mol_type = other DNA
tgtcccccccaccccacagtggggccactagggacaggattggtgacagaaa

SEQ ID NO: 72 - DNA, 52 bp, synthetic construct
  misc_feature 1..52: note = Target oligonucleotide sequence
  source 1..52: mol_type = other DNA
aaaaccctccaccccacagtggggccactagggacaggattggtgacagaaa

SEQ ID NO: 73 - DNA, 52 bp, synthetic construct
  misc_feature 1..52: note = Target oligonucleotide sequence
  source 1..52: mol_type = other DNA
tgtcccctccttttttcagtggggccactagggacaggattggtgacagaaa

SEQ ID NO: 74 - DNA, 23 bp, synthetic construct
  misc_feature 1..23: note = Target oligonucleotide sequence
  source 1..23: mol_type = other DNA
caccggggtggtgcccatcctgg

SEQ ID NO: 75 - DNA, 23 bp, synthetic construct
  misc_feature 1..23: note = Target oligonucleotide sequence
  source 1..23: mol_type = other DNA
ggtgcccatcctggtcgagctgg

SEQ ID NO: 76 - DNA, 23 bp, synthetic construct
  misc_feature 1..23: note = Target oligonucleotide sequence
  source 1..23: mol_type = other DNA
cccatcctggtcgagctggacgg

SEQ ID NO: 77 - DNA, 23 bp, synthetic construct
  misc_feature 1..23: note = Target oligonucleotide sequence
  source 1..23: mol_type = other DNA
ggccacaagttcagcgtgtccgg

SEQ ID NO: 78 - DNA, 23 bp, synthetic construct
  misc_feature 1..23: note = Target oligonucleotide sequence
  source 1..23: mol_type = other DNA
cgcaaataagagctcacctacgg

SEQ ID NO: 79 - DNA, 23 bp, synthetic construct
  misc_feature 1..23: note = Target oligonucleotide sequence
  source 1..23: mol_type = other DNA
ctgaagttcatctgcaccaccgg

SEQ ID NO: 80 - DNA, 23 bp, synthetic construct
  misc_feature 1..23: note = Target oligonucleotide sequence
  source 1..23: mol_type = other DNA
ccggcaagctgcccgtgccctgg

SEQ ID NO: 81 - DNA, 23 bp, synthetic construct
  misc_feature 1..23: note = Target oligonucleotide sequence
  source 1..23: mol_type = other DNA
gaccaggatgggcaccaccccgg

SEQ ID NO: 82 - DNA, 23 bp, synthetic construct
  misc_feature 1..23: note = Target oligonucleotide sequence
  source 1..23: mol_type = other DNA
gccgtccagctcgaccaggatgg

SEQ ID NO: 83 - DNA, 23 bp, synthetic construct
  misc_feature 1..23: note = Target oligonucleotide sequence
  source 1..23: mol_type = other DNA
ggccggacacgctgaacttgtgg

SEQ ID NO: 84 - DNA, 23 bp, synthetic construct
  misc_feature 1..23: note = Target oligonucleotide sequence
  source 1..23: mol_type = other DNA
taacagggtaatgtcgaggccgg

SEQ ID NO: 85 - DNA, 23 bp, synthetic construct
  misc_feature 1..23: note = Target oligonucleotide sequence
  source 1..23: mol_type = other DNA
aggtgagctcttatttgcgtagg

SEQ ID NO: 86 - DNA, 23 bp, synthetic construct
  misc_feature 1..23: note = Target oligonucleotide sequence
  source 1..23: mol_type = other DNA
cttcagggtcagcttgccgtagg

SEQ ID NO: 87 - DNA, 23 bp, synthetic construct
  misc_feature 1..23: note = Target oligonucleotide sequence
  source 1..23: mol_type = other DNA
gggcacgggcagcttgccggtgg

SEQ ID NO: 88 - DNA, 23 bp, synthetic construct
  misc_feature 1..23: note = Target oligonucleotide sequence
  source 1..23: mol_type = other DNA
gagatgatcgccccttcttctgg

SEQ ID NO: 89 - DNA, 20 bp, synthetic construct
  misc_feature 1..20: note = Target oligonucleotide sequence
  source 1..20: mol_type = other DNA
gagatgatcgccccttcttc

SEQ ID NO: 90 - DNA, 20 bp, synthetic construct
  misc_feature 1..20: note = Target oligonucleotide sequence
  source 1..20: mol_type = other DNA
gtgatgaccggccgttcttc

SEQ ID NO: 91 - DNA, 23 bp, synthetic construct
  misc_feature 1..23: note = Target oligonucleotide sequence
  source 1..23: mol_type = other DNA
gtcccctccaccccacagtgggg

SEQ ID NO: 92 - DNA, 23 bp, synthetic construct
  misc_feature 1..23: note = Target oligonucleotide sequence
  source 1..23: mol_type = other DNA
gagatgatcgcccgttcttctgg

SEQ ID NO: 93 - RNA, 20 nt, synthetic construct
  misc_feature 1..20: note = RNA target sequence
  source 1..20: mol_type = other RNA
gtcccctccaccccacagtg

SEQ ID NO: 94 - RNA, 20 nt, synthetic construct
  misc_feature 1..20: note = RNA target sequence
  source 1..20: mol_type = other RNA
gtcccctccaccccacagtc

SEQ ID NO: 95 - RNA, 20 nt, synthetic construct
  misc_feature 1..20: note = RNA target sequence
  source 1..20: mol_type = other RNA
gtcccctccaccccacagag

SEQ ID NO: 96 - RNA, 20 nt, synthetic construct
  misc_feature 1..20: note = RNA target sequence
  source 1..20: mol_type = other RNA
gtcccctccaccccacactg

SEQ ID NO: 97 - RNA, 20 nt, synthetic construct
  misc_feature 1..20: note = RNA target sequence
  source 1..20: mol_type = other RNA
gtcccctccaccccactgtg

SEQ ID NO: 98 - RNA, 20 nt, synthetic construct
  misc_feature 1..20: note = RNA target sequence
  source 1..20: mol_type = other RNA
gtcccctccaccccagagtg

SEQ ID NO: 99 - RNA, 20 nt, synthetic construct
  misc_feature 1..20: note = RNA target sequence
  source 1..20: mol_type = other RNA
gtcccctccacccctcagtg

SEQ ID NO: 100 - RNA, 20 nt, synthetic construct
  misc_feature 1..20: note = RNA target sequence
  source 1..20: mol_type = other RNA
gtcccctccacccgacagtg

SEQ ID NO: 101 - RNA, 20 nt, synthetic construct
  misc_feature 1..20: note = RNA target sequence
  source 1..20: mol_type = other RNA
gtcccctccaccgcacagtg

SEQ ID NO: 102 - RNA, 20 nt, synthetic construct
  misc_feature 1..20: note = RNA target sequence
  source 1..20: mol_type = other RNA
gtcccctccacgccacagtg

SEQ ID NO: 103 - RNA, 20 nt, synthetic construct
  misc_feature 1..20: note = RNA target sequence
  source 1..20: mol_type = other RNA
gtcccctccagcccacagtg

SEQ ID NO: 104 - RNA, 20 nt, synthetic construct
  misc_feature 1..20: note = RNA target sequence
  source 1..20: mol_type = other RNA
gtcccctcctccccacagtg

SEQ ID NO: 105 - RNA, 20 nt, synthetic construct
  misc_feature 1..20: note = RNA target sequence
  source 1..20: mol_type = other RNA
gtcccctcgaccccacagtg

SEQ ID NO: 106 - RNA, 20 nt, synthetic construct
  misc_feature 1..20: note = RNA target sequence
  source 1..20: mol_type = other RNA
gtcccctccaccccacagac

SEQ ID NO: 107 - RNA, 20 nt, synthetic construct
  misc_feature 1..20: note = RNA target sequence
  source 1..20: mol_type = other RNA
gtcccctccaccccactctg

SEQ ID NO: 108 - RNA, 20 nt, synthetic construct
  misc_feature 1..20: note = RNA target sequence
  source 1..20: mol_type = other RNA
gtcccctccacccctgagtg

SEQ ID NO: 109 - RNA, 20 nt, synthetic construct
  misc_feature 1..20: note = RNA target sequence
  source 1..20: mol_type = other RNA
gtcccctccaccggacagtg

SEQ ID NO: 110 - RNA, 20 nt, synthetic construct
  misc_feature 1..20: note = RNA target sequence
  source 1..20: mol_type = other RNA
gtcccctccaggccacagtg

SEQ ID NO: 111 - RNA, 20 nt, synthetic construct
  misc_feature 1..20: note = RNA target sequence
  source 1..20: mol_type = other RNA
gtcccctcgtccccacagtg

SEQ ID NO: 112 - DNA, 23 bp, synthetic construct
  misc_feature 1..23: note = Target oligonucleotide sequence
  source 1..23: mol_type = other DNA
ggggccactagggacaggatggg

SEQ ID NO: 113 - RNA, 20 nt, synthetic construct
  misc_feature 1..20: note = RNA target sequence
  source 1..20: mol_type = other RNA
gagatgatcgccccttcttc

SEQ ID NO: 114 - RNA, 20 nt, synthetic construct
  misc_feature 1..20: note = RNA target sequence
  source 1..20: mol_type = other RNA
gagatgatcgccccttcttg

SEQ ID NO: 115 - RNA, 20 nt, synthetic construct
  misc_feature 1..20: note = RNA target sequence
  source 1..20: mol_type = other RNA
gagatgatcgccccttctac

SEQ ID NO: 116 - RNA, 20 nt, synthetic construct
  misc_feature 1..20: note = RNA target sequence
  source 1..20: mol_type = other RNA
gagatgatcgccccttcatc

SEQ ID NO: 117 - RNA, 20 nt, synthetic construct
  misc_feature 1..20: note = RNA target sequence
  source 1..20: mol_type = other RNA
gagatgatcgccccttgttc

SEQ ID NO: 118 - RNA, 20 nt, synthetic construct
  misc_feature 1..20: note = RNA target sequence
  source 1..20: mol_type = other RNA
gagatgatcgcccctacttc

SEQ ID NO: 119 - RNA, 20 nt, synthetic construct
  misc_feature 1..20: note = RNA target sequence
  source 1..20: mol_type = other RNA
gagatgatcgccccatcttc

SEQ ID NO: 120 - RNA, 20 nt, synthetic construct
  misc_feature 1..20: note = RNA target sequence
  source 1..20: mol_type = other RNA
gagatgatcgcccgttcttc

SEQ ID NO: 121 - RNA, 20 nt, synthetic construct
  misc_feature 1..20: note = RNA target sequence
  source 1..20: mol_type = other RNA
gagatgatcgccgcttcttc

SEQ ID NO: 122 - RNA, 20 nt, synthetic construct
  misc_feature 1..20: note = RNA target sequence
  source 1..20: mol_type = other RNA
gagatgatcgcgccttcttc

SEQ ID NO: 123 - RNA, 20 nt, synthetic construct
  misc_feature 1..20: note = RNA target sequence
  source 1..20: mol_type = other RNA
gagatgatcggcccttcttc

SEQ ID NO: 124 - RNA, 20 nt, synthetic construct
  misc_feature 1..20: note = RNA target sequence
  source 1..20: mol_type = other RNA
gagatgatccccccttcttc

SEQ ID NO: 125 - RNA, 20 nt, synthetic construct
  misc_feature 1..20: note = RNA target sequence
  source 1..20: mol_type = other RNA
gagatgatggccccttcttc

SEQ ID NO: 126 - RNA, 20 nt, synthetic construct
  misc_feature 1..20: note = RNA target sequence
  source 1..20: mol_type = other RNA
gagatgatcgccccttctag

SEQ ID NO: 127 - RNA, 20 nt, synthetic construct
  misc_feature 1..20: note = RNA target sequence
  source 1..20: mol_type = other RNA
gagatgatcgccccttgatc

SEQ ID NO: 128 - RNA, 20 nt, synthetic construct
  misc_feature 1..20: note = RNA target sequence
  source 1..20: mol_type = other RNA
gagatgatcgccccaacttc

SEQ ID NO: 129 - RNA, 20 nt, synthetic construct
  misc_feature 1..20: note = RNA target sequence
  source 1..20: mol_type = other RNA
gagatgatcgccggttcttc

SEQ ID NO: 130 - RNA, 20 nt, synthetic construct
  misc_feature 1..20: note = RNA target sequence
  source 1..20: mol_type = other RNA
gagatgatcgggccttcttc

SEQ ID NO: 131 - RNA, 20 nt, synthetic construct
  misc_feature 1..20: note = RNA target sequence
  source 1..20: mol_type = other RNA
gagatgatgcccccttcttc

SEQ ID NO: 132 - DNA, 23 bp, synthetic construct
  misc_feature 1..23: note = Target oligonucleotide sequence
  source 1..23: mol_type = other DNA
gagatgatcgccccttcttctgg

SEQ ID NO: 133 - RNA, 20 nt, synthetic construct
  misc_feature 1..20: note = RNA target sequence
  source 1..20: mol_type = other RNA
ggggccactagggacaggat

SEQ ID NO: 134 - RNA, 19 nt, synthetic construct
  misc_feature 1..19: note = RNA target sequence
  source 1..19: mol_type = other RNA
gggccactagggacaggat

SEQ ID NO: 135 - RNA, 18 nt, synthetic construct
  misc_feature 1..18: note = RNA target sequence
  source 1..18: mol_type = other RNA
ggccactagggacaggat

SEQ ID NO: 136 - RNA, 17 nt, synthetic construct
  misc_feature 1..17: note = RNA target sequence
  source 1..17: mol_type = other RNA
gccactagggacaggat

SEQ ID NO: 137 - RNA, 20 nt, synthetic construct
  misc_feature 1..20: note = RNA target sequence
  source 1..20: mol_type = other RNA
gagatgatcgccccttcttc

SEQ ID NO: 138 - RNA, 18 nt, synthetic construct
  misc_feature 1..18: note = RNA target sequence
  source 1..18: mol_type = other RNA
gatgatcgccccttcttc

SEQ ID NO: 139 - RNA, 15 nt, synthetic construct
  misc_feature 1..15: note = RNA target sequence
  source 1..15: mol_type = other RNA
gatcgccccttcttc

SEQ ID NO: 140 - RNA, 11 nt, synthetic construct
  misc_feature 1..11: note = RNA target sequence
  source 1..11: mol_type = other RNA
gccccttcttc

SEQ ID NO: 141 - DNA, 21 bp, synthetic construct
  misc_feature 1..21: note = Target oligonucleotide sequence
  source 1..21: mol_type = other DNA
gtcccctccaccccacagtgc

SEQ ID NO: 142 - skipped

SEQ ID NO: 143 - DNA, 14 bp, synthetic construct
  misc_feature 1..14: note = Target oligonucleotide sequence
  source 1..14: mol_type = other DNA
tgtcaaaaaaaccc

SEQ ID NO: 144 - DNA, 14 bp, synthetic construct
  misc_feature 1..14: note = Target oligonucleotide sequence
  source 1..14: mol_type = other DNA
tgtcggggggaccc

SEQ ID NO: 145 - DNA, 14 bp, synthetic construct
  misc_feature 1..14: note = Target oligonucleotide sequence
  source 1..14: mol_type = other DNA
tgtcaaaaaaaccc

SEQ ID NO: 146 - DNA, 14 bp, synthetic construct
  misc_feature 1..14: note = Target oligonucleotide sequence
  source 1..14: mol_type = other DNA
tgtcggggggaccc

SEQ ID NO: 147 - DNA, 14 bp, synthetic construct
  misc_feature 1..14: note = Target oligonucleotide sequence
  source 1..14: mol_type = other DNA
tgtcccccccaccc

SEQ ID NO: 148 - DNA, 14 bp, synthetic construct
  misc_feature 1..14: note = Target oligonucleotide sequence
  source 1..14: mol_type = other DNA
tgtcttttttaccc

SEQ ID NO: 149 - DNA, 14 bp, synthetic construct
  misc_feature 1..14: note = Target oligonucleotide sequence
  source 1..14: mol_type = other DNA
tgtcccccccaccc

SEQ ID NO: 150 - DNA, 14 bp, synthetic construct
  misc_feature 1..14: note = Target oligonucleotide sequence
  source 1..14: mol_type = other DNA
tgtcttttttaccc

SEQ ID NO: 151 - DNA, 23 bp, synthetic construct
  misc_feature 1..23: note = Target oligonucleotide sequence
  source 1..23: mol_type = other DNA
ggatcctgtgtccccgagctggg

SEQ ID NO: 152 - DNA, 23 bp, synthetic construct
  misc_feature 1..23: note = Target oligonucleotide sequence
  source 1..23: mol_type = other DNA
gttaatgtggctctggttctggg

SEQ ID NO: 153 - DNA, 23 bp, synthetic construct
  misc_feature 1..23: note = Target oligonucleotide sequence
  source 1..23: mol_type = other DNA
ggggccactagggacaggattgg

SEQ ID NO: 154 - DNA, 23 bp, synthetic construct
  misc_feature 1..23: note = Target oligonucleotide sequence
  source 1..23: mol_type = other DNA
cttcctagtctcctgatattggg

SEQ ID NO: 155 - DNA, 23 bp, synthetic construct
  misc_feature 1..23: note = Target oligonucleotide sequence
  source 1..23: mol_type = other DNA
tggtcccagctcggggacacagg

SEQ ID NO: 156 - DNA, 23 bp, synthetic construct
  misc_feature 1..23: note = Target oligonucleotide sequence
  source 1..23: mol_type = other DNA
agaaccagagccacattaaccgg

SEQ ID NO: 157 - DNA, 23 bp, synthetic construct
  misc_feature 1..23: note = Target oligonucleotide sequence
  source 1..23: mol_type = other DNA
gtcaccaatcctgtccctagtgg

SEQ ID NO: 158 - DNA, 23 bp, synthetic construct
  misc_feature 1..23: note = Target oligonucleotide sequence
  source 1..23: mol_type = other DNA
agacccaatatcaggagactagg

SEQ ID NO: 159 - DNA, 75 bp, synthetic construct
  misc_feature 1..75: note = Target oligonucleotide sequence
  source 1..75: mol_type = other DNA
gggatcctgtgtccccgagctgggaccaccttatattcccagggccggttaatgtggctctggttctgggtactt

SEQ ID NO: 160 - DNA, 69 bp, synthetic construct
  misc_feature 1..69: note = Target oligonucleotide sequence
  source 1..69: mol_type = other DNA
gggatcctgtgtccccgagctgggaccaccttatattcccagggccggttaatgtggttctgggtactt

SEQ ID NO: 161 - DNA, 113 bp, synthetic construct
  misc_feature 1..113: note = Target oligonucleotide sequence
  source 1..113: mol_type = other DNA
gggatcctgtgtccccgagctgggaccaccttatattcccagggcagggccggttggaccaccttatattcccagggcagggccggttaatgtggctctggttctgggtactt

SEQ ID NO: 162 - DNA, 34 bp, synthetic construct
  misc_feature 1..34: note = Target oligonucleotide sequence
  source 1..34: mol_type = other DNA
gggatcctgtgtccccgtctggttctgggtactt

SEQ ID NO: 163 - DNA, 47 bp, synthetic construct
  misc_feature 1..47: note = Target oligoncleotide sequence
  source 1..47: mol_type = other DNA
gggatcctgtgtccccgagctgggaccaccttatattctgggtactt

SEQ ID NO: 164 - DNA, 17 bp, synthetic construct
  misc_feature 1..17: note = Target oligonucleotide sequence
  source 1..17: mol_type = other DNA
gggatcctgtggtactt

SEQ ID NO: 165 - DNA, 93 bp, synthetic construct
  misc_feature 1..93: note = Target oligonucleotide sequence
  source 1..93: mol_type = other DNA
agggccggttaatgtggctctggttctgggtacttttatctgtcccctccaccccacagtggggccactagggacaggattggtgacagaaaa

SEQ ID NO: 166 - DNA, 83 bp, synthetic construct
  misc_feature 1..83: note = Target oligonucleotide sequence
  source 1..83: mol_type = other DNA
agggccggttaatgaatgtggctctggttctgggtacttttatctgtcccctccaccccacagtggggccactagacagaaaa

SEQ ID NO: 167 - DNA, 76 bp, synthetic construct
  misc_feature 1..76: note = Target oligonucleotide sequence
  source 1..76: mol_type = other DNA
agggccggttaatgtggctctggttctgggtacttttatctgtcccccagtggggccactgattggtgacagaaaa

SEQ ID NO: 168 - DNA, 29 bp, synthetic construct
  misc_feature 1..29: note = Target oligonucleotide sequence
  source 1..29: mol_type = other DNA
agggccggttcaggattggtgacagaaaa

SEQ ID NO: 169 - DNA, 34 bp, synthetic construct
  misc_feature 1..34: note = Target oligonucleotide sequence
  source 1..34: mol_type = other DNA
agggccggttaatgtggcgattggtgacagaaaa

SEQ ID NO: 170 - DNA, 63 bp, synthetic construct
  misc_feature 1..63: note = Target oligonucleotide sequence
  source 1..63: mol_type = other DNA
agggccggttaatgtggctctggttctgggtacttttatctgtccccgattggtgacagaaaa

SEQ ID NO: 171 - DNA, 84 bp, synthetic construct
  misc_feature 1..84: note = Target oligonucleotide sequence
  source 1..84: mol_type = other DNA
agggccggttaatgtggctctggttctgggtacttttatctgtcccctccaccccacagtggggacaggattggtgacagaaaa

SEQ ID NO: 172 - DNA, 27 bp, synthetic construct
  misc_feature 1..27: note = Target oligonucleotide sequence
  source 1..27: mol_type = other DNA
agggccggttaatgtggtgacagaaaa

SEQ ID NO: 173 - DNA, 105 bp, synthetic construct
  misc_feature 1..105: note = Target oligonucleotide sequence
  source 1..105: mol_type = other DNA
agggccggttaatgtggctctggttctgggtacttttatctgtcccctccaccccaggggacagtctgtcccctccaccccagggacaggattggtgacagaaaa

SEQ ID NO: 174 - DNA, 80 bp, synthetic construct
  misc_feature 1..80: note = Target oligonucleotide sequence
  source 1..80: mol_type = other DNA
agggccggttaatgtggctctggttctgggtacttttatctgtcccctccaccactagggacaggattggtgacagaaaa

SEQ ID NO: 175 - DNA, 53 bp, synthetic construct
  misc_feature 1..53: note = Target oligonucleotide sequence
  source 1..53: mol_type = other DNA
cccacagtggggccactagggacaggattggtgacagaaaagccccatacccc

SEQ ID NO: 176 - DNA, 22 bp, synthetic construct
  misc_feature 1..22: note = Target oligonucleotide sequence
  source 1..22: mol_type = other DNA
cccacagtggggccactacccc

SEQ ID NO: 177 - DNA, 96 bp, synthetic construct
  misc_feature 1..96: note = Target oligonucleotide sequence
  source 1..96: mol_type = other DNA
cccacagtggggccactagtagaaaagccccatccttaggcctcccccatccttaggcctcctccttcctagtctcctgatattgggtctaacccc

SEQ ID NO: 178 - DNA, 94 bp, synthetic construct
  misc_feature 1..94: note = Target oligonucleotide sequence
  source 1..94: mol_type = other DNA
cccacagtggggccactagggacaggattggtgacagaaaagccccatccttaggcctcctccttcctagtctcctgatattgggtctaacccc

SEQ ID NO: 179 - DNA, 62 bp, synthetic construct
  misc_feature 1..62: note = Target oligonucleotide sequence
  source 1..62: mol_type = other DNA
cccacagtggggccacccttaggcctcctccttcctagtctcctgatattgggtctaacccc

SEQ ID NO: 180 - DNA, 38 bp, synthetic construct
  misc_feature 1..38: note = Target oligonucleotide sequence
  source 1..38: mol_type = other DNA
cccacagtggggccactagtgatattgggtctaacccc

SEQ ID NO: 181 - DNA, 94 bp, synthetic construct
  misc_feature 1..94: note = target oligonucleotide sequence
  source 1..94: mol_type = other DNA
cccacagtggggccactagggacaggattggtgacaaaaaagccccatccttacgcctcctccttcctagtctcctgatattgggtctaacccc

SEQ ID NO: 182 - DNA, 65 bp, synthetic construct
  misc_feature 1..65: note = Target oligonucleotide sequence
  source 1..65: mol_type = other DNA
cccacagtggggccactagggacaggcctcctccttcctagtctcctgatattgggtctaacccc

SEQ ID NO: 183 - DNA, 102 bp, synthetic construct
  misc_feature 1..102: note = Target oligonucleotide sequence
  source 1..102: mol_type = other DNA
cccacagtggggccactagggacagggggacaggattggtgacagaaaagccccatccttaggcctcctccttcctagtctcctgatattgggtctaacccc

SEQ ID NO: 184 - DNA, 76 bp, synthetic construct
  misc_feature 1..76: note = Target oligonucleotide sequence
  source 1..76: mol_type = other DNA
cccacaggattggtgacagaaaagccccatccttaggcctcctccttcctagtctcctgatattgggtctaacccc